European Patent Application EP 4 257 671 A1, published October 11, 2023. Title: Novel strains of Schizochytrium sp. and method for producing polyunsaturated fatty acid using the same. Applicant: CJ CheilJedang Corporation. The sequence listing filed with the application follows.

SEQUENCE LISTING (3 sequences)

SEQ ID NO: 1 - DNA, 1784 bp, Artificial
  18s rRNA of Shizochytrium sp. CD01-5000
atctggttgatcctgccagtagtcatatgctcgtctcaaagattaagccatgcatgtgtaagtataagcgattgtactgtgagactgcgaacggctcattatatcagtaataatttcttcggtagtttcttttatatggatacctgcagtaattctggaaataatacatgctgtaagagccctgtatggggctgcacttattagattgaagccgattttattggtgaatcatgataattgagcagattgactatttggtcgatgaatcgtttgagtttctgccccatcagttgtcgacggtagtgtattggactacggtgactataacgggtgacggagagttagggctcgactccggagagggagcctgagagacggctaccatatccaaggatagcagcaggcgcgtaaattacccactgtggactccacgaggtagtgacgagaaatatcgatgcgaagcgtgtatgcgttttgctatcggaatgagagcaatgtaaaaccctcatcgaggatcaactggagggcaagtctggtgccagcagccgcggtaattccagctccagaagcatatgctaaagttgttgcagttaaaaagctcgtagttgaatttctggcatgggcgaccggtgctttccctgaatggggattgattgtctgtgttgccttggccatctttttcttttctttataggggagaaatctttcactgtaatcaaagcagagtgttccaagcaggtcgtatgaccggtatgtttattatgggatgataagataggacttgggtgctattttgttggtttgcacgcctgagtaatggttaataggaacagttgggggtattcgtatttaggagctagaggtgaaattcttggatttccgaaagacgaactagagcgaaggcatttaccaagcatgttttcattaatcaagaacgaaagtctggggatcgaagatgattagataccatcgtagtctagaccgtaaacgatgccgacttgcgattgttgggtgcttttttatgggcctcagcagcagcacatgagaaatcaaagtctttgggttccggggggagtatggtcgcaaggctgaaacttaaaggaattgacggaagggcaccaccaggagtggagcctgcggcttaatttgactcaacacgggaaaacttaccaggtccagacataggtaggattgacagattgagagctctttcatgattctatgggtggtggtgcatggccgttcttagttggtggagtgatttgtctggttaattccgttaacgaacgagacctcggcctactaaatagtgcgtggtatggcaacatagtacgttttaacttcttagagggacatgtccggtttacgggcaggaagttcgaggcaataacaggtctgtgatgcccttagatgttctgggccgcacgcgcgctacactgatgggttcatcgggttttaattctgtttttatggaattgagtgcttggtcggaaggcctggctaatccttggaacgctcatcgtgctggggctagatttttgcaattattaatctccaacgaggaattcctagtaaacgcaagtcatcagcttgcattgaatacgtccctgccctttgtacacaccgcccgtcgcacctaccgattgaacggtccgatgaaaccatgggatgtttctgtttggattaatttttggacagaggcagaactcgggtgaatcttattgtttagaggaaggtgaagtcgtaacaaggtttccgtaggtgaacctgcggaaggatcatta

SEQ ID NO: 2 - DNA, 22 bp, Artificial
  18s-001F (primer)
aacctggttgatcctgccagta

SEQ ID NO: 3 - DNA, 25 bp, Artificial
  18s-013R (primer)
ccttgttacgacttcaccttcctct